European Patent Application EP 4 261 288 A1, published October 18, 2023. Title: Method for preparing alpha-branched beta'-hydroxy carbonyl compounds by enzymatic-catalyzed reductive aldol reaction. Applicant: Max-Planck-Gesellschaft zur Foerderung der Wissenschaften e.V. The sequence listing filed with the application follows.

SEQUENCE LISTING (36 sequences)

SEQ ID NO: 1 - protein, 445 aa, Artificial Sequence
  Kitasatospora setae KsCcr crotonyl-CoA carboxylase/reductase
MQEILDAILSGDAASADYAALALPESYRAVTLHKGEERMFDGLASRDKDPRKSLHLDDVPLPELGPGEALVAVMASSVNYNTVWSSIFEPVSTFGFLERYGRLSPLTARHDLPYHVLGSDLAGVVLRTGAGVNAWKPGDEVVAHCLSVELESPDGHNDTMMDPEQRIWGFETNFGGLAQLALVKTNQLLPKPKHLTWEEAASPGLVNSTAYRQLVSRNGAGLKQGDNVLIWGASGGLGSYATQYALAGGATPICVVSSPRKADICRAMGAEAIIDRSAEGYRFWKDEHHQDPREWKRLGGKIREFTGGEDVDIVFEHPGRETFGASVYVTRKGGTIVTCASTSGYMHQYDNRYLWMSLKRIVGSHFANYREAFEANRLVAKGKIHPTLSKVYALEETGQAALDVHHNKHQGKVGVLCLAPREGLGVTDPELRSKHLTKINAFRNV

SEQ ID NO: 2 - protein, 424 aa, Artificial Sequence
  Caulobacter crescentus CcCcr crotonyl-CoA carboxylase/reductase
MTIQTLETTALKDLYEIGEIPPAFHVPKTMYAWSIRKERHGKPTQAMQVEVVPTWEIGEDEVLVLVMAAGVNYNGVWAALGEPISPLDGHKQPFHIAGSDASGIVWKVGAKVKRWKLGDEVVIHCNQDDGDDEECNGGDPMFSSSQRIWGYETPDGSFAQFCRVQSRQLLPRPKHLTWEESACYTLTLATAYRMLFGHKPHELKPGQNVLVWGASGGLGVFATQLAAVAGANAIGVVSSEDKREFVLSMGAKAVLNRGEFNCWGQLPKVNGPEFNDYMKESRKFGKAIWQITGNKDVDMVFEHPGEQTFPVSVFLVKRGGMVVICAGTTGFNLTMDARFLWMRQKRVQGSHFANLMQASAANQLVIDRRVDPCLSEVFPWDQIPAAHEKMLANQHLPGNMAVLVCAQRPGLRTFEEVQELSGAP

SEQ ID NO: 3 - protein, 17 aa, Artificial Sequence
  KsCcr crotonyl-CoA carboxylase/reductase amino acid residues 68-84
EALVAVMASSVNYNTVW

SEQ ID NO: 4 - protein, 17 aa, Artificial Sequence
  CcCcr crotonyl-CoA carboxylase/reductase amino acid residues 61-77
EVLVLVMAAGVNYNGVW

SEQ ID NO: 5 - protein, 33 aa, Artificial Sequence
  KsCcr crotonyl-CoA carboxylase/reductase amino acid residues 113-145
PYHVLGSDLAGVVLRTGAGVNAWKPGDEVVAHC

SEQ ID NO: 6 - protein, 33 aa, Artificial Sequence
  CcCcr crotonyl-CoA carboxylase/reductase amino acid residues 93-125
PFHIAGSDASGIVWKVGAKVKRWKLGDEVVIHC

SEQ ID NO: 7 - protein, 8 aa, Artificial Sequence
  KsCcr crotonyl-CoA carboxylase/reductase amino acid residues 165-172
QRIWGFET

SEQ ID NO: 8 - protein, 8 aa, Artificial Sequence
  CcCcr crotonyl-CoA carboxylase/reductase amino acid residues 146-153
QRIWGYET

SEQ ID NO: 9 - protein, 15 aa, Artificial Sequence
  KsCcr crotonyl-CoA carboxylase/reductase amino acid residues 187-201
QLLPKPKHLTWEEAA

SEQ ID NO: 10 - protein, 15 aa, Artificial Sequence
  CcCcr crotonyl-CoA carboxylase/reductase amino acid residues 168-182
QLLPRPKHLTWEESA

SEQ ID NO: 11 - protein, 6 aa, Artificial Sequence
  KsCcr crotonyl-CoA carboxylase/reductase amino acid residues 208-214
TAYRQL

SEQ ID NO: 12 - protein, 6 aa, Artificial Sequence
  CcCcr crotonyl-CoA carboxylase/reductase amino acid residues 190-195
TAYRML

SEQ ID NO: 13 - protein, 32 aa, Artificial Sequence
  KsCcr crotonyl-CoA carboxylase/reductase amino acid residues 227-258
NVLIWGASGGLGSYATQYALAGGATPICVVSS

SEQ ID NO: 14 - protein, 32 aa, Artificial Sequence
  CcCcr crotonyl-CoA carboxylase/reductase amino acid residues 208-239
NVLVWGASGGLGVFATQLAAVAGANAIGVVSS

SEQ ID NO: 15 - protein, 10 aa, Artificial Sequence
  KsCcr crotonyl-CoA carboxylase/reductase amino acid residues 310-319
DVDIVFEHPG

SEQ ID NO: 16 - protein, 10 aa, Artificial Sequence
  CcCcr crotonyl-CoA carboxylase/reductase amino acid residues 296-305
DVDMVFEHPG

SEQ ID NO: 17 - protein, 6 aa, Artificial Sequence
  KsCcr crotonyl-CoA carboxylase/reductase amino acid residues 363-368
GSHFAN

SEQ ID NO: 18 - protein, 6 aa, Artificial Sequence
  CcCcr crotonyl-CoA carboxylase/reductase amino acid residues 347-354
GSHFAN

SEQ ID NO: 19 - protein, 445 aa, Artificial Sequence
  KsCcr variant His365Asn
MQEILDAILSGDAASADYAALALPESYRAVTLHKGEERMFDGLASRDKDPRKSLHLDDVPLPELGPGEALVAVMASSVNYNTVWSSIFEPVSTFGFLERYGRLSPLTARHDLPYHVLGSDLAGVVLRTGAGVNAWKPGDEVVAHCLSVELESPDGHNDTMMDPEQRIWGFETNFGGLAQLALVKTNQLLPKPKHLTWEEAASPGLVNSTAYRQLVSRNGAGLKQGDNVLIWGASGGLGSYATQYALAGGATPICVVSSPRKADICRAMGAEAIIDRSAEGYRFWKDEHHQDPREWKRLGGKIREFTGGEDVDIVFEHPGRETFGASVYVTRKGGTIVTCASTSGYMHQYDNRYLWMSLKRIVGSNFANYREAFEANRLVAKGKIHPTLSKVYALEETGQAALDVHHNKHQGKVGVLCLAPREGLGVTDPELRSKHLTKINAFRNV

SEQ ID NO: 20 - protein, 445 aa, Artificial Sequence
  KsCcr variant Asn81Leu
MQEILDAILSGDAASADYAALALPESYRAVTLHKGEERMFDGLASRDKDPRKSLHLDDVPLPELGPGEALVAVMASSVNYLTVWSSIFEPVSTFGFLERYGRLSPLTARHDLPYHVLGSDLAGVVLRTGAGVNAWKPGDEVVAHCLSVELESPDGHNDTMMDPEQRIWGFETNFGGLAQLALVKTNQLLPKPKHLTWEEAASPGLVNSTAYRQLVSRNGAGLKQGDNVLIWGASGGLGSYATQYALAGGATPICVVSSPRKADICRAMGAEAIIDRSAEGYRFWKDEHHQDPREWKRLGGKIREFTGGEDVDIVFEHPGRETFGASVYVTRKGGTIVTCASTSGYMHQYDNRYLWMSLKRIVGSHFANYREAFEANRLVAKGKIHPTLSKVYALEETGQAALDVHHNKHQGKVGVLCLAPREGLGVTDPELRSKHLTKINAFRNV

SEQ ID NO: 21 - protein, 445 aa, Artificial Sequence
  KsCcr variant Thr82Asp
MQEILDAILSGDAASADYAALALPESYRAVTLHKGEERMFDGLASRDKDPRKSLHLDDVPLPELGPGEALVAVMASSVNYNDVWSSIFEPVSTFGFLERYGRLSPLTARHDLPYHVLGSDLAGVVLRTGAGVNAWKPGDEVVAHCLSVELESPDGHNDTMMDPEQRIWGFETNFGGLAQLALVKTNQLLPKPKHLTWEEAASPGLVNSTAYRQLVSRNGAGLKQGDNVLIWGASGGLGSYATQYALAGGATPICVVSSPRKADICRAMGAEAIIDRSAEGYRFWKDEHHQDPREWKRLGGKIREFTGGEDVDIVFEHPGRETFGASVYVTRKGGTIVTCASTSGYMHQYDNRYLWMSLKRIVGSHFANYREAFEANRLVAKGKIHPTLSKVYALEETGQAALDVHHNKHQGKVGVLCLAPREGLGVTDPELRSKHLTKINAFRNV

SEQ ID NO: 22 - protein, 445 aa, Artificial Sequence
  KsCcr variant Ser119Ala
MQEILDAILSGDAASADYAALALPESYRAVTLHKGEERMFDGLASRDKDPRKSLHLDDVPLPELGPGEALVAVMASSVNYNTVWSSIFEPVSTFGFLERYGRLSPLTARHDLPYHVLGADLAGVVLRTGAGVNAWKPGDEVVAHCLSVELESPDGHNDTMMDPEQRIWGFETNFGGLAQLALVKTNQLLPKPKHLTWEEAASPGLVNSTAYRQLVSRNGAGLKQGDNVLIWGASGGLGSYATQYALAGGATPICVVSSPRKADICRAMGAEAIIDRSAEGYRFWKDEHHQDPREWKRLGGKIREFTGGEDVDIVFEHPGRETFGASVYVTRKGGTIVTCASTSGYMHQYDNRYLWMSLKRIVGSHFANYREAFEANRLVAKGKIHPTLSKVYALEETGQAALDVHHNKHQGKVGVLCLAPREGLGVTDPELRSKHLTKINAFRNV

SEQ ID NO: 23 - protein, 445 aa, Artificial Sequence
  KsCcr variant Phe170Ala
MQEILDAILSGDAASADYAALALPESYRAVTLHKGEERMFDGLASRDKDPRKSLHLDDVPLPELGPGEALVAVMASSVNYNTVWSSIFEPVSTFGFLERYGRLSPLTARHDLPYHVLGSDLAGVVLRTGAGVNAWKPGDEVVAHCLSVELESPDGHNDTMMDPEQRIWGAETNFGGLAQLALVKTNQLLPKPKHLTWEEAASPGLVNSTAYRQLVSRNGAGLKQGDNVLIWGASGGLGSYATQYALAGGATPICVVSSPRKADICRAMGAEAIIDRSAEGYRFWKDEHHQDPREWKRLGGKIREFTGGEDVDIVFEHPGRETFGASVYVTRKGGTIVTCASTSGYMHQYDNRYLWMSLKRIVGSHFANYREAFEANRLVAKGKIHPTLSKVYALEETGQAALDVHHNKHQGKVGVLCLAPREGLGVTDPELRSKHLTKINAFRNV

SEQ ID NO: 24 - protein, 445 aa, Artificial Sequence
  KsCcr variant Glu171Ala
MQEILDAILSGDAASADYAALALPESYRAVTLHKGEERMFDGLASRDKDPRKSLHLDDVPLPELGPGEALVAVMASSVNYNTVWSSIFEPVSTFGFLERYGRLSPLTARHDLPYHVLGSDLAGVVLRTGAGVNAWKPGDEVVAHCLSVELESPDGHNDTMMDPEQRIWGFATNFGGLAQLALVKTNQLLPKPKHLTWEEAASPGLVNSTAYRQLVSRNGAGLKQGDNVLIWGASGGLGSYATQYALAGGATPICVVSSPRKADICRAMGAEAIIDRSAEGYRFWKDEHHQDPREWKRLGGKIREFTGGEDVDIVFEHPGRETFGASVYVTRKGGTIVTCASTSGYMHQYDNRYLWMSLKRIVGSHFANYREAFEANRLVAKGKIHPTLSKVYALEETGQAALDVHHNKHQGKVGVLCLAPREGLGVTDPELRSKHLTKINAFRNV

SEQ ID NO: 25 - protein, 445 aa, Artificial Sequence
  KsCcr variant Ile167Ala
MQEILDAILSGDAASADYAALALPESYRAVTLHKGEERMFDGLASRDKDPRKSLHLDDVPLPELGPGEALVAVMASSVNYNTVWSSIFEPVSTFGFLERYGRLSPLTARHDLPYHVLGSDLAGVVLRTGAGVNAWKPGDEVVAHCLSVELESPDGHNDTMMDPEQRAWGFETNFGGLAQLALVKTNQLLPKPKHLTWEEAASPGLVNSTAYRQLVSRNGAGLKQGDNVLIWGASGGLGSYATQYALAGGATPICVVSSPRKADICRAMGAEAIIDRSAEGYRFWKDEHHQDPREWKRLGGKIREFTGGEDVDIVFEHPGRETFGASVYVTRKGGTIVTCASTSGYMHQYDNRYLWMSLKRIVGSHFANYREAFEANRLVAKGKIHPTLSKVYALEETGQAALDVHHNKHQGKVGVLCLAPREGLGVTDPELRSKHLTKINAFRNV

SEQ ID NO: 26 - protein, 445 aa, Artificial Sequence
  KsCcr variant Met356Ala
MQEILDAILSGDAASADYAALALPESYRAVTLHKGEERMFDGLASRDKDPRKSLHLDDVPLPELGPGEALVAVMASSVNYNTVWSSIFEPVSTFGFLERYGRLSPLTARHDLPYHVLGSDLAGVVLRTGAGVNAWKPGDEVVAHCLSVELESPDGHNDTMMDPEQRIWGFETNFGGLAQLALVKTNQLLPKPKHLTWEEAASPGLVNSTAYRQLVSRNGAGLKQGDNVLIWGASGGLGSYATQYALAGGATPICVVSSPRKADICRAMGAEAIIDRSAEGYRFWKDEHHQDPREWKRLGGKIREFTGGEDVDIVFEHPGRETFGASVYVTRKGGTIVTCASTSGYMHQYDNRYLWASLKRIVGSHFANYREAFEANRLVAKGKIHPTLSKVYALEETGQAALDVHHNKHQGKVGVLCLAPREGLGVTDPELRSKHLTKINAFRNV

SEQ ID NO: 27 - protein, 445 aa, Artificial Sequence
  KsCcr variant Met356Val
MQEILDAILSGDAASADYAALALPESYRAVTLHKGEERMFDGLASRDKDPRKSLHLDDVPLPELGPGEALVAVMASSVNYNTVWSSIFEPVSTFGFLERYGRLSPLTARHDLPYHVLGSDLAGVVLRTGAGVNAWKPGDEVVAHCLSVELESPDGHNDTMMDPEQRIWGFETNFGGLAQLALVKTNQLLPKPKHLTWEEAASPGLVNSTAYRQLVSRNGAGLKQGDNVLIWGASGGLGSYATQYALAGGATPICVVSSPRKADICRAMGAEAIIDRSAEGYRFWKDEHHQDPREWKRLGGKIREFTGGEDVDIVFEHPGRETFGASVYVTRKGGTIVTCASTSGYMHQYDNRYLWVSLKRIVGSHFANYREAFEANRLVAKGKIHPTLSKVYALEETGQAALDVHHNKHQGKVGVLCLAPREGLGVTDPELRSKHLTKINAFRNV

SEQ ID NO: 28 - DNA, 32 bp, Artificial Sequence
  I176A Forward Primer 5'->3'
gacccagagcagcgcgcctggggcttcgaaac

SEQ ID NO: 29 - protein, 424 aa, Artificial Sequence
  CcCcr variant C125P/I148A/F352G
MTIQTLETTALKDLYEIGEIPPAFHVPKTMYAWSIRKERHGKPTQAMQVEVVPTWEIGEDEVLVLVMAAGVNYNGVWAALGEPISPLDGHKQPFHIAGSDASGIVWKVGAKVKRWKLGDEVVIHPNQDDGDDEECNGGDPMFSSSQRAWGYETPDGSFAQFCRVQSRQLLPRPKHLTWEESACYTLTLATAYRMLFGHKPHELKPGQNVLVWGASGGLGVFATQLAAVAGANAIGVVSSEDKREFVLSMGAKAVLNRGEFNCWGQLPKVNGPEFNDYMKESRKFGKAIWQITGNKDVDMVFEHPGEQTFPVSVFLVKRGGMVVICAGTTGFNLTMDARFLWMRQKRVQGSHGANLMQASAANQLVIDRRVDPCLSEVFPWDQIPAAHEKMLANQHLPGNMAVLVCAQRPGLRTFEEVQELSGAP

SEQ ID NO: 30 - protein, 14 aa, Artificial Sequence
  KsCcr crotonyl-CoA carboxylase/reductase amino acid residues 355-368
WMSLKRIVGSHFAN

SEQ ID NO: 31 - protein, 14 aa, Artificial Sequence
  CcCcr crotonyl-CoA carboxylase/reductase amino acid residues 339-354
WMRQKRVQGSHFAN

SEQ ID NO: 32 - DNA, 32 bp, Artificial Sequence
  I176A Reverse Primer 5'->3'
gtttcgaagccccaggcgcgctgctctgggtc

SEQ ID NO: 33 - DNA, 34 bp, Artificial Sequence
  M356A Forward Primer 5'->3'
caaccgttacctgtgggcgtccctgaaacgtatc

SEQ ID NO: 34 - DNA, 34 bp, Artificial Sequence
  M356A Reverse Primer 5'->3'
gatacgtttcagggacgcccacaggtaacggttg

SEQ ID NO: 35 - DNA, 26 bp, Artificial Sequence
  M356V Forward Primer 5'->3'
ccgttacctgtgggtgtccctgaaac

SEQ ID NO: 36 - DNA, 26 bp, Artificial Sequence
  M356V Reverse Primer 5'->3'
gtttcagggacacccacaggtaacgg